European Patent Application EP 4 289 962 A2, published December 13, 2023. Title: COMPOSITIONS COMPRISING POLYSACCHARIDES OR EXTRACT DERIVED FROM LACTOBACILLUS PLANTARUM. Applicant: Neoregen Biotech. The sequence listing filed with the application follows.

SEQUENCE LISTING (30 sequences)

SEQ ID NO: 1 - DNA, 20 bp, Artificial Sequence
  mouse PPAR gamma forward primer
ttcagaagtgccttgctgtg

SEQ ID NO: 2 - DNA, 21 bp, Artificial Sequence
  mouse PPAR gamma reverse primer
gctggtcgatatcactggaga

SEQ ID NO: 3 - DNA, 20 bp, Artificial Sequence
  mouse C/EBP alpha forward primer
ggtgcgtctaagatgaggga

SEQ ID NO: 4 - DNA, 20 bp, Artificial Sequence
  mouse C/EBP alpha reverse primer
ccccctactcggtaggaaaa

SEQ ID NO: 5 - DNA, 23 bp, Artificial Sequence
  mouse FABP4 forward primer
aaggtgaagagcatcataaccct

SEQ ID NO: 6 - DNA, 23 bp, Artificial Sequence
  mouse FABP4 reverse primer
tcacgcctttcataacacattcc

SEQ ID NO: 7 - DNA, 21 bp, Artificial Sequence
  mouse LPL forward primer
atggatggacggtaacgggaa

SEQ ID NO: 8 - DNA, 23 bp, Artificial Sequence
  mouse LPL reverse primer
cccgatacaaccagtctactaca

SEQ ID NO: 9 - DNA, 22 bp, Artificial Sequence
  mouse FAS forward primer
atccggaacgagaacacgatct

SEQ ID NO: 10 - DNA, 23 bp, Artificial Sequence
  mouse FAS reverse primer
agagacgtgtcactcctggactt

SEQ ID NO: 11 - DNA, 20 bp, Artificial Sequence
  mouse GPDH forward primer
atggctggcaagaaagtctg

SEQ ID NO: 12 - DNA, 21 bp, Artificial Sequence
  mouse GPDH reverse primer
cgtgctgagtgttgatgatct

SEQ ID NO: 13 - DNA, 21 bp, Artificial Sequence
  mouse CD36 forward primer
agatgacgtggcaaagaacag

SEQ ID NO: 14 - DNA, 23 bp, Artificial Sequence
  mouse CD36 reverse primer
ccttggctagataacgaactctg

SEQ ID NO: 15 - DNA, 21 bp, Artificial Sequence
  mouse GAPDH forward primer
aggtcggtgtgaacggatttg

SEQ ID NO: 16 - DNA, 23 bp, Artificial Sequence
  mouse GAPDH reverse primer
tgtagaccatgtagttgaggtca

SEQ ID NO: 17 - DNA, 22 bp, Artificial Sequence
  human PPAR gamma forward  primer
accaaagtgcaatcaaagtgga

SEQ ID NO: 18 - DNA, 21 bp, Artificial Sequence
  human PPAR gamma reverse primer
atgagggagttggaaggctct

SEQ ID NO: 19 - DNA, 21 bp, Artificial Sequence
  human C/EBP alpha forward primer
aacacgaagcacgatcagtcc

SEQ ID NO: 20 - DNA, 21 bp, Artificial Sequence
  human C/EBP alpha reverse primer
ctcattttggcaagtatccga

SEQ ID NO: 21 - DNA, 20 bp, Artificial Sequence
  human FABP4 forward primer
actgggccaggaatttgacg

SEQ ID NO: 22 - DNA, 19 bp, Artificial Sequence
  human FABP4 reverse primer
ctcgtggaagtgacgcctt

SEQ ID NO: 23 - DNA, 21 bp, Artificial Sequence
  human Leptin forward primer
tgccttccagaaacgtgatcc

SEQ ID NO: 24 - DNA, 21 bp, Artificial Sequence
  human Leptin reverse primer
ctctgtggagtagcctgaagc

SEQ ID NO: 25 - DNA, 23 bp, Artificial Sequence
  human GPDH forward primer
ctatacagcatcctccagcacaa

SEQ ID NO: 26 - DNA, 19 bp, Artificial Sequence
  human GPDH reverse primer
ggccctcgtagcacacctt

SEQ ID NO: 27 - DNA, 23 bp, Artificial Sequence
  human CD36 forward primer
ctttggcttaatgagactgggac

SEQ ID NO: 28 - DNA, 21 bp, Artificial Sequence
  human CD36 reverse primer
gcaacaaacatcaccacacca

SEQ ID NO: 29 - DNA, 20 bp, Artificial Sequence
  human GAPDH forward primer
tggactccacgacgtactca

SEQ ID NO: 30 - DNA, 20 bp, Artificial Sequence
  human GAPDH reverse primer
acatgttccaatatgattcc